European Patent Specification EP 4 004 231 B1, published November 12, 2025. Title: SINGLE CELL CHROMATIN IMMUNOPRECIPITATION SEQUENCING ASSAY. Applicant: Becton, Dickinson and Company Song, Hye-Won. The sequence listing filed with the application follows.

SEQUENCE LISTING (3 sequences)

SEQ ID NO: 1 - DNA, 11 bp, Artificial Sequence
  Synthetic oligonucleotide
  misc_feature (8)..(11): n is a, c, g, or t
tttttttnnnn

SEQ ID NO: 2 - DNA, 11 bp, Artificial Sequence
  Synthetic oligonucleotide
  misc_feature (1)..(5): n is a, c, g, or t
nnnnnaaaaaa

SEQ ID NO: 3 - DNA, 12 bp, Artificial Sequence
  Synthetic oligonucleotide
  misc_feature (8)..(12): n is a, c, g, or t
tttttttnnnnn